European Patent Application EP 4 379 064 A1, published June 5, 2024. Title: Diagnostic methods and diagnostic assay comprising detection of lncDNAs. Applicant: Ruprecht-Karls-Universität Heidelberg. Application EP. The sequence listing filed with the application follows.

SEQUENCE LISTING (33 sequences)

SEQ ID NO: 1 - DNA, 852 bp, Homo sapiens
  source 1..852: mol_type = other DNA
tcgttccaatgagaatgaaggctgaggtgtgcgcctttttttttttttccttcttagtcgtgtgtacatcattgggaatggagggaaataaatgactggatggtcgctgctttttaagtttcaaattgacattccagacaagcggtgcctgagcccgtgcctgtcttcagatcttcacagcacagttcctgggaaggtggagccaccagcctctccttgtcctggaggctggaagtgcaaaaggaaggtgtcggcaagatcgtttttttctgagagctctctccttggcttgcagatggcagcctgctcctggcacagtcttttctctactcatgcccaaagttacggaggacccagcaaccatctcctgcagcccctggaaacctcttgactcttctgtgatgtccccagtgatccagcagccctggccttcttttgatggcttgaacatttggtcttcattgaacagtttgtatattggaaacttgccagcctccatccacattccaacctccgtctgcatccctcgaataactgggagatgaaacaggaagctctatgacacacttgatcgaatatgacagacaccgaaaatcacgactcagccccctccagcacctctacctgttgcccgccgatcacagccggaatgcagctgaaagattccctggggcctggttccaaccgcccactgtggactctgaggcctctgcatttgcgggtggtctgcctgtgatattttggtcatgggctggtctggtcggtttcccatttgtctggccagtctctatgtgtcttaatcccttgtccttcattaaaagcaaaactaaagaaaacagaaaaaaaaaaaaa

SEQ ID NO: 2 - DNA, 732 bp, Homo sapiens
  source 1..732: mol_type = other DNA
tcgttccaatgagaatgaaggctgaggtgtgcgcctttttttttttttccttcttagtcgtgtgtacatcattgggaatggagggaaataaatgactggatggtcgctgctttttaagtttcaaattgacattccagacaagcggtgcctgagcccgtgcctgtcttcagatcttcacagcacagttcctgggaaggtggagccaccagcctctccttgactcatgcccaaagttacggaggacccagcaaccatctcctgcagcccctggaaacctcttgactcttctgtgatgtccccagtgatccagcagccctggccttcttttgatggcttgaacatttggtcttcattgaacagtttgtatattggaaacttgccagcctccatccacattccaacctccgtctgcatccctcgaataactgggagatgaaacaggaagctctatgacacacttgatcgaatatgacagacaccgaaaatcacgactcagccccctccagcacctctacctgttgcccgccgatcacagccggaatgcagctgaaagattccctggggcctggttccaaccgcccactgtggactctgaggcctctgcatttgcgggtggtctgcctgtgatattttggtcatgggctggtctggtcggtttcccatttgtctggccagtctctatgtgtcttaatcccttgtccttcattaaaagcaaaactaaagaaaacagaa

SEQ ID NO: 3 - DNA, 3887 bp, Homo sapiens
  source 1..3887: mol_type = other DNA
acaagtatgaagagaatgtcgggagaggaagtggtggctatgagtcagcatgagtcatctcgttccaatgagaatgaaggctgaggtgtgcgccttttttttttttccttcttagtcgtgtgtacatcattgggaatggagggaaataaatgactggatggtcgctgctttttaagtttcaaattgacattccagacaagcggtgcctgagcccgtgcctgtcttcagatcttcacagcacagttcctgggaaggtggagccaccagcctctccctgacaagcaaagtggatcagcaaaggctgcagtcaccagcatcttttccaaccttaatgaactgtatcctcaaaagaacactatcagactggtaagacaagcattattgtcccacttcacagatgaagagcttgggggccctgtggatgtgtaggagagtcggccttcctttttataggccttttgctgagctcagaggacagagcagaagacaaagccgaatgcagccctaagcagacactatcccagcccaaggagctatgcagacagctcctgcctagaggagaaacaattctctccttcagccaggcatgtggcacagaggtgaacaggaaatgcttagggagacagttcacagatatatatgtacttcacagggcacaatttaatccataaatcaatcatggatcaccgctaaagaaaacaaaatatgctgccactaatttgccaccaccctgtgagcatgattggatgatgtttattttgattaggagattgctccatttataaatcttcaatacatcctgtccccctaaaacggcatctgggtcttttgagggttaaaaaaaaaaaaaagtgaaattggatgagggatgagagctggacttctgtgtgtcccggggtccctggatccacagcctggtgcctagcatcagttaagcccacgctggggtcgcatcacatcccgcaaagccacgtgctctgtgaggccaacaggagccccgccgggtggaccagctggaatctcagagagcgccgactctgaaactacccggctctgcagaagcacgctgggcccaggggcttctagactgacagctccatttatcaactacctattggttttaaaaattggagtgtcttttccgcgttgactgattttggctctaagagatgtcgctggtcatttcagagtgactgaacctcccctctaacagatcccgggaattgttttcaggaaaggtaaaaggcagccttttctgtcacaacacaacgctgagccggcagcctggctctgtcaggatctggggctcccgcgcccgagaagcccagcctcgccggcggccaagttcaccgcgaggccccgcgctgcctgcgctgcgctcccggacccgcaccgaccgcagcgcgcgccgccggtgcttctcccaccccagcctggaagctgcctccctccgcctatgcctgcaggataagaagcccgaggaggcggagcatggaactcgacagttaaaacatttaagagagaaaacctagtgtcttgctggcctgaaatcgagtacgcagcccggggtgatcagggtctcccggcccggatgtgtgagacttgcttcccctgggcaataggcgatacgatgctttaggaggaaggtgtctctccctcctaagccccggaggggagaacttccaaagacagaaaaccacaggcttcctggcacagagctttccctttatcagctaaagcagaatcttttctggccttaacctggccccttcctctaactgcaggcagagaggcagacagaaaagcacttgctgaaacacaaagttttgttctgtcctcaacgaactgtctagagctgattgctgatagtcgtggtgcattatgccttcctggttttcatttaattgggcaccacgctgcctttcaagacgccttaaaggaaccaacaaccaaatccaagagagctggacagaccattgaacacacagtaggctgtgtctcgtggctttcgttgtctggtgcctcaaagaaaacaccagaaagattgtttctaagctagagccaccccagattgcttaaagtgcaaagctcactgctgttgggggtacccttgtgagacactggaaagctggttttaccgtggccctatgaagaggaagactgaaatttagacagtaatacctttactaggattggaaaagatttggttaatgacagccctgtcatttctaaaacccattatcactgtatgagagattcctttgcgctgcatcctcgacagtgcttcctaaggctctgccgacttccagttctggaacaagatggttaaactcatttttccctgctctgctcctctaaatacaactaagtaccttggaaactattcagcagacaatgataaagggctctgaaagctagaagaaaaggtgtacttgcaagaaacctcaggacttgagtaacagcaacatgaacaatccatttcacagatgaagaaacagactcagtgagcacgtgatcacttctcacaactaatggagccaagattctgtccttatggctccagagacctcttttttttcccactgtaccacaacactcaccaggactggagtgccacctatgacctcattgcataatggatggcttgtcctcaaatgggcccggtcttggacgagcctgaggatgtctacaagtggaagaaaagaagccactggagcagaaggtggggaggataaaatttggagcaagattctcaaggaagcaacaagatcctaagatcttgttctcactagagaataatttctacattatgcccaggttcttctgagctatgaaggggcccagatttaagggctatttttgacaccctaaatgtgctgagacaagtcattaaggtggtcctgccaggacacagccatctaaagcagcaatctgcttcttgccagaaaatctcgtgcctctgcagagccttttccagaatgaaccacaccatgctgaggaaaggagaaagagactacctactgcatttctgtcactcgctgaaaaggacactctgtcagaaaatcttctagcaaacttcaaagggcaaaatcaccccttgttactgataaagcccagagagcttcagcagctaacattccctggacagggcacagcaaggatttgaacctaggtcagtctggccagaacacccacaagctttccttaactcagtgtgctatctccccacgactaggtcactactgctttataatcacctttgtagccaccagtggattttgctcatcagtatttttcaggcaattgatactttagatattcagctgcaagacgtatgcagttttcattgacatcttttggagaaactgacaaacctggacttgacttaatgcctttggaaccttccaagatgttatataactctagatagaaggctgggcctccatgatgtcaggaatgttgcattcttatttccccatagataaacccatttgtccacaaagtcaaggagtcaggcagaggcccttgccatggggctttttaggataaagcaacaagcctggactttgctctacaacagggttttgcatagggagtggtatgaccagatccctcaagaaagaaagcttagagaccaggccagagtccactgcagtagcccagtcaagagaggatggtgacttggacttgtagtagagccagttagaatgaaagaaattgacacattcagaaatggttttagagatagagtcaaactggacctgataaagaactagagaagcggagtgaggataaagagaagagccatgactgactcggaagattttgtcttgaaaaacttgagaactcaagacagagtgaaataaaatcacatgtgggaaaaatct

SEQ ID NO: 4 - DNA, 1137 bp, Homo sapiens
  source 1..1137: mol_type = other DNA
ctcatttttctactgctcgtggatttacgcgcacgttggaaccgaagagagctctgttgttgcaatgttcagcccacaagagcttactggtgaaggaatgggacaagacccatctttatgcaaagccagcgttacagtaatgttccagcatctcataatctatcctggggaattcagctgcctcccagggtgaatacaggtattcctgatgacagtctgcctctatcttacagagcagcttgttgctatataccattgaaaagccttcagagctgagaggtactactaaccaataacctgcttggctcaaagggccagcaccttctctctaaagcccaagaggagtttgaggaaaactaggtgtctgtgttcactccaggctgaagttacaggtctgagcaaataaggtgtataaaaaatggaatctgtcttggaggacatcagaaggtgaattttccaagttcttggacaacctagctgttgaaaagctttctgggtttggggggtatttcagatgtaccttaaagtgttagcagacacagattaagacactgggagccaatgaaacagcagttgagggtttgctgtgtatcacatttctgtattttatcacccccttcctgcaacattatttatctggaatctacctgcccttttgttttttagatacaagggcttggttttgttacccaggctggtttcaaggccatagctttaagagatcctctcaccacagatttccaaagtgctgggattgcaggtgtgattcatggcacccagactttgctgcctttcttacatgatccaggcccagaacccaaactcaggcactgtatagatgaccactttcgtaaactactgacctagcttgttgccaattgttgattgaacttcccataactccacttcgtgtctgttcctctgtatacagccaccttctgttcccgtcatgagcctttaggtctccatttgcatattgcaaatactatgttccatgtaggtagctcattcagggccttgctcttcacttcaaaaaaggttcccttgaggactggctgtcaatttgtgttgctgtgttggttgttgatgaaaataataaaatgattgattacatagtcctgtttaaaaaaaaaaaaa

SEQ ID NO: 5 - DNA, 1535 bp, Homo sapiens
  source 1..1535: mol_type = other DNA
ctcatttttctactgctcgtggtaagtggcttcgtggtctttatagctgttactcttttgtactttgtctttttcttttattttcttttgagcgattgtgcgaacatagcatagcacgcactatgccttctgtgttgtagctgcctggccagggcgactggcggataaggtcttgtgcgtggcctcgaggcttaaaagtagcagtggggctttgtgaaggacaaaatggcgatggcgggccgtgtaggtcccccttcctatgatgaggaccttttcacagacctgtactgagctccgtgaggataaataactctgaggagatgggccctgcaagcctcttgcttagccgtctgttcagaaaatagcgttttcgaaatgccctgagttgacctaatgtcttattgggctcctgtctgcaggatttacgcgcacgttggaaccgaagagagctctgttgttgcaatgttcagcccacaagagcttactggtgaaggaatgggacaagacccatctttatgcaaagccagcgttacagtaatgttccagcatctcataatctatcctggggaattcagctgcctcccagggtgaatacaggtattcctgatgacagtctgcctctatcttacagagcagcttgttgctatataccattgaaaagccttcagagctgagaggtactactaaccaataacctgcttggctcaaagggccagcaccttctctctaaagcccaagaggagtttgaggaaaactaggtgtctgtgttcactccaggctgaagttacaggtctgagcaaataaggtgtataaaaaatggaatctgtcttggaggacatcagaaggtgaattttccaagttcttggacaacctagctgttgaaaagctttctgggtttggggggtatttcagatgtaccttaaagtgttagcagacacagattaagacactgggagccaatgaaacagcagttgagggtttgctgtgtatcacatttctgtattttatcacccccttcctgcaacattatttatctggaatctacctgcccttttgttttttagatacaagggcttggttttgttacccaggctggtttcaaggccatagctttaagagatcctctcaccacagatttccaaagtgctgggattgcaggtgtgattcatggcacccagactttgctgcctttcttacatgatccaggcccagaacccaaactcaggcactgtatagatgaccactttcgtaaactactgacctagcttgttgccaattgttgattgaacttcccataactccacttcgtgtctgttcctctgtatacagccaccttctgttcccgtcatgagcctttaggtctccatttgcatattgcaaatactatgttccatgtaggtagctcattcagggccttgctcttcacttcaaaaaaggttcccttgaggactggctgtcaatttgtgttgctgtgttggttgttgatgaaaataataaaatgattgattacatagtcctgtttaaaaaaaaaaaaa

SEQ ID NO: 6 - DNA, 1527 bp, Homo sapiens
  source 1..1527: mol_type = other DNA
ctcatttttctactgctcgtggtaagtggcttcgtggtctttatagctgttactcttttgtactttgtctttttcttttattttcttttgagcgattgtgcgaacatagcatagcacgcactatgccttctgtgttgtagctgcctggccagggcgactggcggataaggtcttgtgcgtggcctcgaggcttaaaagtagcagtggggctttgtgaaggacaaaatggcgatggcgggccgtgtaggtcccccttcctatgatgaggaccttttcacagacctgtactgagctccgtgaggataaataactctgaggagatgggccctgcaagcctcttgcttagccgtctgttcagaaaatagcgttttcgaaatgccctgagttgacctaatgtcttattgggctcctgtctgcaggatttacgcgcacgttggaaccgaagagagctctgttgttgcacccacaagagcttactggtgaaggaatgggacaagacccatctttatgcaaagccagcgttacagtaatgttccagcatctcataatctatcctggggaattcagctgcctcccagggtgaatacaggtattcctgatgacagtctgcctctatcttacagagcagcttgttgctatataccattgaaaagccttcagagctgagaggtactactaaccaataacctgcttggctcaaagggccagcaccttctctctaaagcccaagaggagtttgaggaaaactaggtgtctgtgttcactccaggctgaagttacaggtctgagcaaataaggtgtataaaaaatggaatctgtcttggaggacatcagaaggtgaattttccaagttcttggacaacctagctgttgaaaagctttctgggtttggggggtatttcagatgtaccttaaagtgttagcagacacagattaagacactgggagccaatgaaacagcagttgagggtttgctgtgtatcacatttctgtattttatcacccccttcctgcaacattatttatctggaatctacctgcccttttgttttttagatacaagggcttggttttgttacccaggctggtttcaaggccatagctttaagagatcctctcaccacagatttccaaagtgctgggattgcaggtgtgattcatggcacccagactttgctgcctttcttacatgatccaggcccagaacccaaactcaggcactgtatagatgaccactttcgtaaactactgacctagcttgttgccaattgttgattgaacttcccataactccacttcgtgtctgttcctctgtatacagccaccttctgttcccgtcatgagcctttaggtctccatttgcatattgcaaatactatgttccatgtaggtagctcattcagggccttgctcttcacttcaaaaaaggttcccttgaggactggctgtcaatttgtgttgctgtgttggttgttgatgaaaataataaaatgattgattacatagtcctgtttaaaaaaaaaaaaa

SEQ ID NO: 7 - DNA, 918 bp, Homo sapiens
  source 1..918: mol_type = other DNA
ctcatttttctactgctcgtggatttacgcgcacgttggaaccgaagagagctctgttgttgcaatgttcagcccacaagagcttactggtgaaggaatgggacaagacccatctttatgcaaagccagcgttacagtaatgttccagcatctcataatctatcctggggaattcagctgcctcccagggtgaatacaggtattcctgatgacagtctgcctctatcttacagagcagcttgttgctatataccattgaaaagccttcagagctgagaggtactactaaccaataacctgcttggctcaaagggccagcaccttctctctaaagcccaagaggagtttgaggaaaactaggtgtctgtgttcactccaggctgaagttacaggtctgagcaaataaggtgtataaaaaatggaatctgtcttggaggacatcagaagatacaagggcttggttttgttacccaggctggtttcaaggccatagctttaagagatcctctcaccacagatttccaaagtgctgggattgcaggtgtgattcatggcacccagactttgctgcctttcttacatgatccaggcccagaacccaaactcaggcactgtatagatgaccactttcgtaaactactgacctagcttgttgccaattgttgattgaacttcccataactccacttcgtgtctgttcctctgtatacagccaccttctgttcccgtcatgagcctttaggtctccatttgcatattgcaaatactatgttccatgtaggtagctcattcagggccttgctcttcacttcaaaaaaggttcccttgaggactggctgtcaatttgtgttgctgtgttggttgttgatgaaaataataaaatgattgattacatagtcctgtttaaaaaaaaaaaaa

SEQ ID NO: 8 - DNA, 1316 bp, Homo sapiens
  source 1..1316: mol_type = other DNA
ctcatttttctactgctcgtggtaagtggcttcgtggtctttatagctgttactcttttgtactttgtctttttcttttattttcttttgagcgattgtgcgaacatagcatagcacgcactatgccttctgtgttgtagctgcctggccagggcgactggcggataaggtcttgtgcgtggcctcgaggcttaaaagtagcagtggggctttgtgaaggacaaaatggcgatggcgggccgtgtaggtcccccttcctatgatgaggaccttttcacagacctgtactgagctccgtgaggataaataactctgaggagatgggccctgcaagcctcttgcttagccgtctgttcagaaaatagcgttttcgaaatgccctgagttgacctaatgtcttattgggctcctgtctgcaggatttacgcgcacgttggaaccgaagagagctctgttgttgcaatgttcagcccacaagagcttactggtgaaggaatgggacaagacccatctttatgcaaagccagcgttacagtaatgttccagcatctcataatctatcctggggaattcagctgcctcccagggtgaatacaggtattcctgatgacagtctgcctctatcttacagagcagcttgttgctatataccattgaaaagccttcagagctgagaggtactactaaccaataacctgcttggctcaaagggccagcaccttctctctaaagcccaagaggagtttgaggaaaactaggtgtctgtgttcactccaggctgaagttacaggtctgagcaaataaggtgtataaaaaatggaatctgtcttggaggacatcagaagatacaagggcttggttttgttacccaggctggtttcaaggccatagctttaagagatcctctcaccacagatttccaaagtgctgggattgcaggtgtgattcatggcacccagactttgctgcctttcttacatgatccaggcccagaacccaaactcaggcactgtatagatgaccactttcgtaaactactgacctagcttgttgccaattgttgattgaacttcccataactccacttcgtgtctgttcctctgtatacagccaccttctgttcccgtcatgagcctttaggtctccatttgcatattgcaaatactatgttccatgtaggtagctcattcagggccttgctcttcacttcaaaaaaggttcccttgaggactggctgtcaatttgtgttgctgtgttggttgttgatgaaaataataaaatgattgattacatagtcctgtttaaaaaaaaaaaaa

SEQ ID NO: 9 - DNA, 1135 bp, Homo sapiens
  source 1..1135: mol_type = other DNA
gtatttccgccggcgcgaaacgagcgtagcttccttgtcgtgtggcctcagtccttcgccgtccctcgccgtccttcgccatcgcacgccaccgcaccccatctctcgaaatctgcagacatcttgatttttcccacgctgtctgtcaggtctccgccgccactcgacgccagggcgccgggccttgtgggctgtgctgcacctcggacggcttcgcaccagccagcgccctctctctcctgcagcactctgatctgcaccccctgaggggcttccactgtccgcggggtgagaatgcccctgggagtgtcacatgactgccgccccatgtgtgtgagaggcgtcctctgggagagcatggatcctgaggtcccaggattgtcagctgacctctgtcctgtgtgcccagtggccccaggtgacgtgtcttcaagaagaggctgagctgcggtgcttgtaaggcagggtctcattctgtcacccaggctggagtgcagtggtgcaatgatggctcactgcagcctcgacctgggctcaagtgatcctccacctcagcttcctgagtagctgggaccacagagtcatgtgctgttcctggggcttggatgatgtaggggaagcaaggtgaaagtggtatcccgtggttccacgttctgtcctgctgtggggctgtccctcacatgctttcagtggctgttgcagaggaagagcctccggaaatctgcgtgggtctcagccttagatccaaggacagtccaaggaagtcctaagaccatggagttggtgatctgggatctgggtttgctgatatttctcaccgtgaatctcttggtggtgtttgtgggcacgagaggggcagagaatggagagtgaggctaccacatgaagcgtcaccagagctgctccctgctgcctgctcagagcaccccggatccactgttcaatctgcacaagattcggggtccagacatgggagacttcagctgcctcagaggaccgtggacagggaaggccagcctcgcatccctctgtccatgcctggaatgactttaataaccaagagttttatttttgaatttgtagctgtcgttcactttttacccacccattcaataaaccttacagaattgctcca

SEQ ID NO: 10 - DNA, 1209 bp, Homo sapiens
  source 1..1209: mol_type = other DNA
gtatttccgccggcgcgaaacgagcgtagcttccttgtcgtgtggcctcagtccttcgccgtccctcgccgtccttcgccatcgcacgccaccgcaccccatctctcgaaatctgcagacatcttgatttttcccacgctgtctgtcaggtctccgccgccactcgacgccagggcgccgggtgagtccacagcagggcgcatggtcggctccactctcaccatcgggggaaactgaggccccggggaaggcggccagagaggtcaggccctgtccttggtgcagtgtctcgtcctctttgccggagtgagccccccaggattcgcgtgtcctcgggaaagacactggcaggccttgtgggctgtgctgcacctcggacggcttcgcaccagccagcgccctctctctcctgcagcactctgatctgcaccccctgaggggcttccactgtccgcggggtgagaatgcccctgggagtgtcacatgactgccgccccatgtgtgtgagaggcgtcctctgggagagcatggatcctgaggtcccaggattgtcagctgacctctgtcctgtgtgcccagtggccccaggtgacgtgtcttcaagaagaggctgagctgcggtgcttgtaagagtcatgtgctgttcctggggcttggatgatgtaggggaagcaaggtgaaagtggtatcccgtggttccacgttctgtcctgctgtggggctgtccctcacatgctttcagtggctgttgcagaggaagagcctccggaaatctgcgtgggtaaagtctcagccttagatccaaggacagtccaaggaagtcctaagaccatggagttggtgatctgggatctgggtttgctgatatttctcaccgtgaatctcttggtggtgtttgtgggcacgagaggggcagagaatggagagtgaggctaccacatgaagcgtcaccagagctgctccctgctgcctgctcagagcaccccggatccactgttcaatctgcacaagattcggggtccagacatgggagacttcagctgcctcagaggaccgtggacagggaaggccagcctcgcatccctctgtccatgcctggaatgactttaataaccaagagttttatttttgaatttgtagctgtcgttcactttttacccacccattcaataaaccttacagaattgctccaaaaaaaaaaaaaaaaaa

SEQ ID NO: 11 - DNA, 945 bp, Homo sapiens
  source 1..945: mol_type = other DNA
gtatttccgccggcgcgaaacgagcgtagcttccttgtcgtgtggcctcagtccttcgccgtccctcgccgtccttcgccatcgcacgccaccgcaccccatctctcgaaatctgcagacatcttgatttttcccacgctgtctgtcaggtctccgccgccactcgacgccagggcgccgggccttgtgggctgtgctgcacctcggacggcttcgcaccagccagcgccctctctctcctgcagcactctgatctgcaccccctgaggggcttccactgtccgcggggtgagaatgcccctgggagtgtcacatgactgccgccccatgtgtgtgagaggcgtcctctgggagagcatggatcctgaggtcccaggattgtcagctgacctctgtcctgtgtgcccagtggccccaggtgacgtgtcttcaagaagaggctgagctgcggtgcttgtaagatgggtctgctgtgtgcagaggctccatgggatgtgttgtcttcatagtagcagggcgctggaccatgggtccgcaaggtctcagccttagatccaaggacagtccaaggaagtcctaagaccatggagttggtgatctgggatctgggtttgctgatatttctcaccgtgaatctcttggtggtgtttgtgggcacgagaggggcagagaatggagagtgaggctaccacatgaagcgtcaccagagctgctccctgctgcctgctcagagcaccccggatccactgttcaatctgcacaagattcggggtccagacatgggagacttcagctgcctcagaggaccgtggacagggaaggccagcctcgcatccctctgtccatgcctggaatgactttaataaccaagagttttatttttgaatttgtagctgtcgttcactttttacccacccattcaataaaccttacagaattgctcca

SEQ ID NO: 12 - DNA, 1301 bp, Homo sapiens
  source 1..1301: mol_type = other DNA
gtatttccgccggcgcgaaacgagcgtagcttccttgtcgtgtggcctcagtccttcgccgtccctcgccgtccttcgccatcgcacgccaccgcaccccatctctcgaaatctgcagacatcttgatttttcccacgctgtctgtcaggtctccgccgccactcgacgccagggcgccgggtgagtccacagcagggcgcatggtcggctccactctcaccatcgggggaaactgaggccccggggaaggcggccagagaggtcaggccctgtccttggtgcagtgtctcgtcctctttgccggagtgagccccccaggattcgcgtgtcctcgggaaagacactggcaggccttgtgggctgtgctgcacctcggacggcttcgcaccagccagcgccctctctctcctgcagcactctgatctgcaccccctgaggggcttccactgtccgcggggtgagaatgcccctgggagtgtcacatgactgccgccccatgtgtgtgagaggcgtcctctgggagagcatggatcctgaggtcccaggattgtcagctgacctctgtcctgtgtgcccagtggccccaggtgacgtgtcttcaagaagaggctgagctgcggtgcttgtaagggtctcattctgtcacccaggctggagtgcagtggtgcaatgatggctcactgcagcctcgacctgggctcaagtgatcctccacctcagcttcctgagtagctgggaccacagagtcatgtgctgttcctggggcttggatgatgtaggggaagcaaggtgaaagtggtatcccgtggttccacgttctgtcctgctgtggggctgtccctcacatgctttcagtggctgttgcagaggaagagcctccggaaatctgcgtgggtctcagccttagatccaaggacagtccaaggaagtcctaagaccatggagttggtgatctgggatctgggtttgctgatatttctcaccgtgaatctcttggtggtgtttgtgggcacgagaggggcagagaatggagagtgaggctaccacatgaagcgtcaccagagctgctccctgctgcctgctcagagcaccccggatccactgttcaatctgcacaagattcggggtccagacatgggagacttcagctgcctcagaggaccgtggacagggaaggccagcctcgcatccctctgtccatgcctggaatgactttaataaccaagagttttatttttgaatttgtagctgtcgttcactttttacccacccattcaataaaccttacagaattgctcca

SEQ ID NO: 13 - DNA, 1022 bp, Homo sapiens
  source 1..1022: mol_type = other DNA
gtatttccgccggcgcgaaacgagcgtagcttccttgtcgtgtggcctcagtccttcgccgtccctcgccgtccttcgccatcgcacgccaccgcaccccatctctcgaaatctgcagacatcttgatttttcccacgctgtctgtcaggtctccgccgccactcgacgccagggcgccgggccttgtgggctgtgctgcacctcggacggcttcgcaccagccagcgccctctctctcctgcagcactctgatctgcaccccctgaggggcttccactgtccgcggggtgagaatgcccctgggagtgtcacatgactgccgccccatgtgtgtgagaggcgtcctctgggagagcatggatcctgaggtcccaggattgtcagctgacctctgtcctgtgtgcccagtggccccaggtgacgtgtcttcaagaagaggctgagctgcggtgcttgtaagagtcatgtgctgttcctggggcttggatgatgtaggggaagcaaggtgaaagtggtatcccgtggttccacgttctgtcctgctgtggggctgtccctcacatgctttcagtggctgttgcagaggaagagcctccggaaatctgcgtgggtaaagtctcagccttagatccaaggacagtccaaggaagtcctaagaccatggagttggtgatctgggatctgggtttgctgatatttctcaccgtgaatctcttggtggtgtttgtgggcacgagaggggcagagaatggagagtgaggctaccacatgaagcgtcaccagagctgctccctgctgcctgctcagagcaccccggatccactgttcaatctgcacaagattcggggtccagacatgggagacttcagctgcctcagaggaccgtggacagggaaggccagcctcgcatccctctgtccatgcctggaatgactttaataaccaagagttttatttttgaatttgtagctgtcgttcactttttacccacccattcaataaaccttacagaattgctcca

SEQ ID NO: 14 - DNA, 1034 bp, Homo sapiens
  source 1..1034: mol_type = other DNA
gtatttccgccggcgcgaaacgagcgtagcttccttgtcgtgtggcctcagtccttcgccgtccctcgccgtccttcgccatcgcacgccaccgcaccccatctctcgaaatctgcagacatcttgatttttcccacgctgtctgtcaggtctccgccgccactcgacgccagggcgccgggccttgtgggctgtgctgcacctcggacggcttcgcaccagccagcgccctctctctcctgcagcactctgatctgcaccccctgaggggcttccactgtccgcggggtgagaatgcccctgggagtgtcacatgactgccgccccatgtgtgtgagaggcgtcctctgggagagcatggatcctgaggtcccaggattgtcagctgacctctgtcctgtgtgcccagtggccccaggtgacgtgtcttcaagaagaggctgagctgcggtgcttgtaagagtcatgtgctgttcctggggcttggatgatgtaggggaagcaaggtgaaagtggtatcccgtggttccacgttctgtcctgctgtggggctgtccctcacatgctttcagtggctgttgcagaggaagagcctccggaaatctgcgtgggtctcagccttagatccaaggacagtccaaggaagtcctaagaccatggagttggtgatctgggatctgggtttgctgatatttctcaccgtgaatctcttggtggtgtttgtgggcacgagaggggcagagaatggagagtgaggctaccacatgaagcgtcaccagagctgctccctgctgcctgctcagagcaccccggatccactgttcaatctgcacaagattcggggtccagacatgggagacttcagctgcctcagaggaccgtggacagggaaggccagcctcgcatccctctgtccatgcctggaatgactttaataaccaagagttttatttttgaatttgtagctgtcgttcactttttacccacccattcaataaaccttacagaattgctccaaaaaaaaaaaaaaaaaa

SEQ ID NO: 15 - DNA, 954 bp, Homo sapiens
  source 1..954: mol_type = other DNA
gtatttccgccggcgcgaaacgagcgtagcttccttgtcgtgtggcctcagtccttcgccgtccctcgccgtccttcgccatcgcacgccaccgcaccccatctctcgaaatctgcagacatcttgatttttcccacgctgtctgtcaggtctccgccgccactcgacgccagggcgccgggccttgtgggctgtgctgcacctcggacggcttcgcaccagccagcgccctctctctcctgcagcactctgatctgcaccccctgaggggcttccactgtccgcggggtgagaatgcccctgggagtgtcacatgactgccgccccatgtgtgtgagaggcgtcctctgggagagcatggatcctgaggtcccaggaacatcccgagagccaagttcccagatgccagccaagggccatctgacctgttttgaatctcaatttcctgatacagaaaacaaaggattgtcagctgacctctgtcctgtgtgcccagtggccccaggtgacgtgtcttcaagaagaggctgagctgcggtgcttgtaaggtctcagccttagatccaaggacagtccaaggaagtcctaagaccatggagttggtgatctgggatctgggtttgctgatatttctcaccgtgaatctcttggtggtgtttgtgggcacgagaggggcagagaatggagagtgaggctaccacatgaagcgtcaccagagctgctccctgctgcctgctcagagcaccccggatccactgttcaatctgcacaagattcggggtccagacatgggagacttcagctgcctcagaggaccgtggacagggaaggccagcctcgcatccctctgtccatgcctggaatgactttaataaccaagagttttatttttgaatttgtagctgtcgttcactttttacccacccattcaataaaccttacagaattgctcca

SEQ ID NO: 16 - DNA, 1204 bp, Homo sapiens
  source 1..1204: mol_type = other DNA
gtatttccgccggcgcgaaacgagcgtagcttccttgtcgtgtggcctcagtccttcgccgtccctcgccgtccttcgccatcgcacgccaccgcaccccatctctcgaaatctgcagacatcttgatttttcccacgctgtctgtcaggtctccgccgccactcgacgccagggcgccgggtgagtccacagcagggcgcatggtcggctccactctcaccatcgggggaaactgaggccccggggaaggcggccagagaggtcaggccctgtccttggtgcagtgtctcgtcctctttgccggagtgagccccccaggattcgcgtgtcctcgggaaagacactggcaggccttgtgggctgtgctgcacctcggacggcttcgcaccagccagcgccctctctctcctgcagcactctgatctgcaccccctgaggggcttccactgtccgcggggtgagaatgcccctgggagtgtcacatgactgccgccccatgtgtgtgagaggcgtcctctgggagagcatggatcctgaggtcccaggattgtcagctgacctctgtcctgtgtgcccagtggccccaggtgacgtgtcttcaagaagaggctgagctgcggtgcttgtaagagtcatgtgctgttcctggggcttggatgatgtaggggaagcaaggtgaaagtggtatcccgtggttccacgttctgtcctgctgtggggctgtccctcacatgctttcagtggctgttgcagaggaagagcctccggaaatctgcgtgggtctcagccttagatccaaggacagtccaaggaagtcctaagaccatggagttggtgatctgggatctgggtttgctgatatttctcaccgtgaatctcttggtggtgtttgtgggcacgagaggggcagagaatggagagtgaggctaccacatgaagcgtcaccagagctgctccctgctgcctgctcagagcaccccggatccactgttcaatctgcacaagattcggggtccagacatgggagacttcagctgcctcagaggaccgtggacagggaaggccagcctcgcatccctctgtccatgcctggaatgactttaataaccaagagttttatttttgaatttgtagctgtcgttcactttttacccacccattcaataaaccttacagaattgctccaaaaaaaaaaaaaaaaaa

SEQ ID NO: 17 - DNA, 1115 bp, Homo sapiens
  source 1..1115: mol_type = other DNA
gtatttccgccggcgcgaaacgagcgtagcttccttgtcgtgtggcctcagtccttcgccgtccctcgccgtccttcgccatcgcacgccaccgcaccccatctctcgaaatctgcagacatcttgatttttcccacgctgtctgtcaggtctccgccgccactcgacgccagggcgccgggtgagtccacagcagggcgcatggtcggctccactctcaccatcgggggaaactgaggccccggggaaggcggccagagaggtcaggccctgtccttggtgcagtgtctcgtcctctttgccggagtgagccccccaggattcgcgtgtcctcgggaaagacactggcaggccttgtgggctgtgctgcacctcggacggcttcgcaccagccagcgccctctctctcctgcagcactctgatctgcaccccctgaggggcttccactgtccgcggggtgagaatgcccctgggagtgtcacatgactgccgccccatgtgtgtgagaggcgtcctctgggagagcatggatcctgaggtcccaggattgtcagctgacctctgtcctgtgtgcccagtggccccaggtgacgtgtcttcaagaagaggctgagctgcggtgcttgtaagatgggtctgctgtgtgcagaggctccatgggatgtgttgtcttcatagtagcagggcgctggaccatgggtccgcaaggtctcagccttagatccaaggacagtccaaggaagtcctaagaccatggagttggtgatctgggatctgggtttgctgatatttctcaccgtgaatctcttggtggtgtttgtgggcacgagaggggcagagaatggagagtgaggctaccacatgaagcgtcaccagagctgctccctgctgcctgctcagagcaccccggatccactgttcaatctgcacaagattcggggtccagacatgggagacttcagctgcctcagaggaccgtggacagggaaggccagcctcgcatccctctgtccatgcctggaatgactttaataaccaagagttttatttttgaatttgtagctgtcgttcactttttacccacccattcaataaaccttacagaattgctcca

SEQ ID NO: 18 - DNA, 1146 bp, Homo sapiens
  source 1..1146: mol_type = other DNA
gtatttccgccggcgcgaaacgagcgtagcttccttgtcgtgtggcctcagtccttcgccgtccctcgccgtccttcgccatcgcacgccaccgcaccccatctctcgaaatctgcagacatcttgatttttcccacgctgtctgtcaggtctccgccgccactcgacgccagggcgccgggccttgtgggctgtgctgcacctcggacggcttcgcaccagccagcgccctctctctcctgcagcactctgatctgcaccccctgaggggcttccactgtccgcggggtgagaatgcccctgggagtgtcacatgactgccgccccatgtgtgtgagaggcgtcctctgggagagcatggatcctgaggtcccaggaacatcccgagagccaagttcccagatgccagccaagggccatctgacctgttttgaatctcaatttcctgatacagaaaacaaaggattgtcagctgacctctgtcctgtgtgcccagtggccccaggtgacgtgtcttcaagaagaggctgagctgcggtgcttgtaagggtctcattctgtcacccaggctggagtgcagtggtgcaatgatggctcactgcagcctcgacctgggctcaagtgatcctccacctcagcttcctgagtagctgggaccacagatgggtctgctgtgtgcagaggctccatgggatgtgttgtcttcatagtagcagggcgctggaccatgggtccgcaaggtctcagccttagatccaaggacagtccaaggaagtcctaagaccatggagttggtgatctgggatctgggtttgctgatatttctcaccgtgaatctcttggtggtgtttgtgggcacgagaggggcagagaatggagagtgaggctaccacatgaagcgtcaccagagctgctccctgctgcctgctcagagcaccccggatccactgttcaatctgcacaagattcggggtccagacatgggagacttcagctgcctcagaggaccgtggacagggaaggccagcctcgcatccctctgtccatgcctggaatgactttaataaccaagagttttatttttgaatttgtagctgtcgttcactttttacccacccattcaataaaccttacagaattgctcca

SEQ ID NO: 19 - DNA, 1037 bp, Homo sapiens
  source 1..1037: mol_type = other DNA
gtatttccgccggcgcgaaacgagcgtagcttccttgtcgtgtggcctcagtccttcgccgtccctcgccgtccttcgccatcgcacgccaccgcaccccatctctcgaaatctgcagacatcttgatttttcccacgctgtctgtcaggtctccgccgccactcgacgccagggcgccgggtgagtccacagcagggcgcatggtcggctccactctcaccatcgggggaaactgaggccccggggaaggcggccagagaggtcaggccctgtccttggtgcagtgtctcgtcctctttgccggagtgagccccccaggattcgcgtgtcctcgggaaagacactggcaggccttgtgggctgtgctgcacctcggacggcttcgcaccagccagcgccctctctctcctgcagcactctgatctgcaccccctgaggggcttccactgtccgcggggtgagaatgcccctgggagtgtcacatgactgccgccccatgtgtgtgagaggcgtcctctgggagagcatggatcctgaggtcccaggattgtcagctgacctctgtcctgtgtgcccagtggccccaggtgacgtgtcttcaagaagaggctgagctgcggtgcttgtaaggtctcagccttagatccaaggacagtccaaggaagtcctaagaccatggagttggtgatctgggatctgggtttgctgatatttctcaccgtgaatctcttggtggtgtttgtgggcacgagaggggcagagaatggagagtgaggctaccacatgaagcgtcaccagagctgctccctgctgcctgctcagagcaccccggatccactgttcaatctgcacaagattcggggtccagacatgggagacttcagctgcctcagaggaccgtggacagggaaggccagcctcgcatccctctgtccatgcctggaatgactttaataaccaagagttttatttttgaatttgtagctgtcgttcactttttacccacccattcaataaaccttacagaattgctcca

SEQ ID NO: 20 - DNA, 884 bp, Homo sapiens
  source 1..884: mol_type = other DNA
gtatttccgccggcgcgaaacgagcgtagcttccttgtcgtgtggcctcagtccttcgccgtccctcgccgtccttcgccatcgcacgccaccgcaccccatctctcgaaatctgcagacatcttgatttttcccacgctgtctgtcaggtctccgccgccactcgacgccagggcgccgggccttgtgggctgtgctgcacctcggacggcttcgcaccagccagcgccctctctctcctgcagcactctgatctgcaccccctgaggggcttccactgtccgcggggtgagaatgcccctgggagtgtcacatgactgccgccccatgtgtgtgagaggcgtcctctgggagagcatggatcctgaggtcccaggattgtcagctgacctctgtcctgtgtgcccagtggccccaggtgacgtgtcttcaagaagaggctgagctgcggtgcttgtaaggtctcagccttagatccaaggacagtccaaggaagtcctaagaccatggagttggtgatctgggatctgggtttgctgatatttctcaccgtgaatctcttggtggtgtttgtgggcacgagaggggcagagaatggagagtgaggctaccacatgaagcgtcaccagagctgctccctgctgcctgctcagagcaccccggatccactgttcaatctgcacaagattcggggtccagacatgggagacttcagctgcctcagaggaccgtggacagggaaggccagcctcgcatccctctgtccatgcctggaatgactttaataaccaagagttttatttttgaatttgtagctgtcgttcactttttacccacccattcaataaaccttacagaattgctccaaaaaaaaaaaaaaaaaa

SEQ ID NO: 21 - DNA, 1059 bp, Homo sapiens
  source 1..1059: mol_type = other DNA
gtatttccgccggcgcgaaacgagcgtagcttccttgtcgtgtggcctcagtccttcgccgtccctcgccgtccttcgccatcgcacgccaccgcaccccatctctcgaaatctgcagacatcttgatttttcccacgctgtctgtcaggtctccgccgccactcgacgccagggcgccgggccttgtgggctgtgctgcacctcggacggcttcgcaccagccagcgccctctctctcctgcagcactctgatctgcaccccctgaggggcttccactgtccgcggggtgagaatgcccctgggagtgtcacatgactgccgccccatgtgtgtgagaggcgtcctctgggagagcatggatcctgaggtcccaggattgtcagctgacctctgtcctgtgtgcccagtggccccaggtgacgtgtcttcaagaagaggctgagctgcggtgcttgtaagggtctcattctgtcacccaggctggagtgcagtggtgcaatgatggctcactgcagcctcgacctgggctcaagtgatcctccacctcagcttcctgagtagctgggaccacagatgggtctgctgtgtgcagaggctccatgggatgtgttgtcttcatagtagcagggcgctggaccatgggtccgcaaggtctcagccttagatccaaggacagtccaaggaagtcctaagaccatggagttggtgatctgggatctgggtttgctgatatttctcaccgtgaatctcttggtggtgtttgtgggcacgagaggggcagagaatggagagtgaggctaccacatgaagcgtcaccagagctgctccctgctgcctgctcagagcaccccggatccactgttcaatctgcacaagattcggggtccagacatgggagacttcagctgcctcagaggaccgtggacagggaaggccagcctcgcatccctctgtccatgcctggaatgactttaataaccaagagttttatttttgaatttgtagctgtcgttcactttttacccacccattcaataaaccttacagaattgctcca

SEQ ID NO: 22 - DNA, 1002 bp, Homo sapiens
  source 1..1002: mol_type = other DNA
gtatttccgccggcgcgaaacgagcgtagcttccttgtcgtgtggcctcagtccttcgccgtccctcgccgtccttcgccatcgcacgccaccgcaccccatctctcgaaatctgcagacatcttgatttttcccacgctgtctgtcaggtctccgccgccactcgacgccagggcgccgggccttgtgggctgtgctgcacctcggacggcttcgcaccagccagcgccctctctctcctgcagcactctgatctgcaccccctgaggggcttccactgtccgcggggtgagaatgcccctgggagtgtcacatgactgccgccccatgtgtgtgagaggcgtcctctgggagagcatggatcctgaggtcccaggattgtcagctgacctctgtcctgtgtgcccagtggccccaggtgacgtgtcttcaagaagaggctgagctgcggtgcttgtaaggcagggtctcattctgtcacccaggctggagtgcagtggtgcaatgatggctcactgcagcctcgacctgggctcaagtgatcctccacctcagcttcctgagtagctgggaccacaggtctcagccttagatccaaggacagtccaaggaagtcctaagaccatggagttggtgatctgggatctgggtttgctgatatttctcaccgtgaatctcttggtggtgtttgtgggcacgagaggggcagagaatggagagtgaggctaccacatgaagcgtcaccagagctgctccctgctgcctgctcagagcaccccggatccactgttcaatctgcacaagattcggggtccagacatgggagacttcagctgcctcagaggaccgtggacagggaaggccagcctcgcatccctctgtccatgcctggaatgactttaataaccaagagttttatttttgaatttgtagctgtcgttcactttttacccacccattcaataaaccttacagaattgctccaaaaaaaaaaaaaaaaaa

SEQ ID NO: 23 - DNA, 20 bp, synthetic construct
  source 1..20: mol_type = other DNA
atgcccaaagttacggagga

SEQ ID NO: 24 - DNA, 20 bp, synthetic construct
  source 1..20: mol_type = other DNA
tattcgagggatgcagacgg

SEQ ID NO: 25 - DNA, 20 bp, synthetic construct
  source 1..20: mol_type = other DNA
agcgtagcttccttgtcgtg

SEQ ID NO: 26 - DNA, 20 bp, synthetic construct
  source 1..20: mol_type = other DNA
gagacctgacagacagcgtg

SEQ ID NO: 27 - DNA, 20 bp, synthetic construct
  source 1..20: mol_type = other DNA
gtcattaaggtggtcctgcc

SEQ ID NO: 28 - DNA, 21 bp, synthetic construct
  source 1..21: mol_type = other DNA
agtgtccttttcagcgagtga

SEQ ID NO: 29 - DNA, 20 bp, synthetic construct
  source 1..20: mol_type = other DNA
acgttggaaccgaagagagc

SEQ ID NO: 30 - DNA, 20 bp, synthetic construct
  source 1..20: mol_type = other DNA
gcagctgaattccccaggat

SEQ ID NO: 31 - DNA, 97 bp, synthetic construct
  source 1..97: mol_type = other DNA
tgctgttgacagtgagcgcccgctgcatttataaagaatatagtgaagccacagatgtatattctttataaatgcagcggatgcctactgcctcgga

SEQ ID NO: 32 - DNA, 18 bp, synthetic construct
  source 1..18: mol_type = other DNA
gagcgcccgctgcattta

SEQ ID NO: 33 - DNA, 20 bp, synthetic construct
  source 1..20: mol_type = other DNA
gtaggcatccgctgcattta